European Patent Application EP 4 289 942 A1, published December 13, 2023. Title: Methods for Generation of Retinal Outer Layer Cells from Stem Cells and Composition for Preventing or Treating Retinal Diseases Comprising Cells Thereby Generated. Applicant: S-Biomedics. The sequence listing filed with the application follows.

SEQUENCE LISTING (8 sequences)

SEQ ID NO: 1 - DNA, 20 bp, Artificial Sequence
  Rhodopsin F primer
cacaggatgcaatttggagg

SEQ ID NO: 2 - DNA, 20 bp, Artificial Sequence
  Rhodopsin R primer
ccttctgtgtggtggctgac

SEQ ID NO: 3 - DNA, 20 bp, Artificial Sequence
  beta III tubulin F primer
caacagcacggccatccagg

SEQ ID NO: 4 - DNA, 21 bp, Artificial Sequence
  beta III tubulin R primer
cttggggccctgggcctccga

SEQ ID NO: 5 - DNA, 21 bp, Artificial Sequence
  Nestin F primer
cagctggcgcacctcaagatg

SEQ ID NO: 6 - DNA, 23 bp, Artificial Sequence
  Nestin R primer
agggaagttgggctcaggactgg

SEQ ID NO: 7 - DNA, 20 bp, Artificial Sequence
  GAPDH F primer
accacagtccatgccatcac

SEQ ID NO: 8 - DNA, 20 bp, Artificial Sequence
  GAPDH R primer
tccaccaccctgttgctgta